European Patent Application EP 4 289 427 A1, published December 13, 2023. Title: New compounds for use for treating cancer. Applicant: ANAGENESIS BIOTECHNOLOGIES. The sequence listing filed with the application follows.

SEQUENCE LISTING (10 sequences)

SEQ ID NO: 1 - DNA, 20 bp, artificial
  primer
aacccaagcacgtatcaggg

SEQ ID NO: 2 - DNA, 20 bp, artificial
  primer
gagtgttgggggcatcatca

SEQ ID NO: 3 - DNA, 20 bp, artificial
  primer
catttgctccaaactggcgt

SEQ ID NO: 4 - DNA, 20 bp, artificial
  primer
ttgttctggatcgccccttc

SEQ ID NO: 5 - DNA, 20 bp, artificial
  primer
tccagagagaggaagccgaa

SEQ ID NO: 6 - DNA, 20 bp, artificial
  primer
aaggtcaagacgtgccagag

SEQ ID NO: 7 - DNA, 21 bp, artificial
  primer
ggatgttccctccacagttca

SEQ ID NO: 8 - DNA, 20 bp, artificial
  primer
tgtccgcctaaagccatgtt

SEQ ID NO: 9 - DNA, 20 bp, artificial
  primer
tcaagaccaacggactcctg

SEQ ID NO: 10 - DNA, 20 bp, artificial
  primer
ggtccccacttccctagttg